European Patent Application EP 4 620 483 A1, published September 24, 2025. Title: PHARMACEUTICAL COMPOSITION COMPRISING ANTI-RANKL-NGF BISPECIFIC ANTIBODIES. Applicant: JIANGSU HENGRUI PHARMACEUTICALS CO., LTD. Application IB PCT/CN2023/131913, filed November 16, 2023. The sequence listing filed with the application follows.

SEQUENCE LISTING (41 sequences)

SEQ ID NO: 1 - protein, 5 aa, synthetic construct
SYAMS

SEQ ID NO: 2 - protein, 17 aa, synthetic construct
GITGSGGSTYYADSVKG

SEQ ID NO: 3 - protein, 13 aa, synthetic construct
DPGTTSIMSWFDP

SEQ ID NO: 4 - protein, 12 aa, synthetic construct
RASQSVRGRYLA

SEQ ID NO: 5 - protein, 7 aa, synthetic construct
GASSRAT

SEQ ID NO: 6 - protein, 9 aa, synthetic construct
QQYGSSPRT

SEQ ID NO: 7 - protein, 122 aa, synthetic construct
EVQLLESGGGLVQPGGSLRLSCAASGFTFSSYAMSWVRQAPGKGLEWVSGITGSGGSTYYADSVKGRFTISRDNSKNTLYLQMNSLRAEDTAVYYCVKDPGTTSIMSWFDPWGQGTLVTVSS

SEQ ID NO: 8 - protein, 108 aa, synthetic construct
EIVLTQSPGTLSLSPGERATLSCRASQSVRGRYLAWYQQKPGQAPRLLIYGASSRATGIPDRFSGSGSGTDFTLTISRLEPEDFAVFYCQQYGSSPRTFGQGTKVEIK

SEQ ID NO: 9 - protein, 327 aa, synthetic construct
ASTKGPSVFPLAPCSRSTSESTAALGCLVKDYFPEPVTVSWNSGALTSGVHTFPAVLQSSGLYSLSSVVTVPSSSLGTKTYTCNVDHKPSNTKVDKRVESKYGPPCPPCPAPEFLGGPSVFLFPPKPKDTLMISRTPEVTCVVVDVSQEDPEVQFNWYVDGVEVHNAKTKPREEQFNSTYRVVSVLTVLHQDWLNGKEYKCKVSNKGLPSSIEKTISKAKGQPREPQVYTLPPSQEEMTKNQVSLTCLVKGFYPSDIAVEWESNGQPENNYKTTPPVLDSDGSFFLYSRLTVDKSRWQEGNVFSCSVMHEALHNHYTQKSLSLSLGK

SEQ ID NO: 10 - protein, 107 aa, synthetic construct [sequence omitted]

SEQ ID NO: 11 - protein, 449 aa, synthetic construct
EVQLLESGGGLVQPGGSLRLSCAASGFTFSSYAMSWVRQAPGKGLEWVSGITGSGGSTYYADSVKGRFTISRDNSKNTLYLQMNSLRAEDTAVYYCVKDPGTTSIMSWFDPWGQGTLVTVSSASTKGPSVFPLAPCSRSTSESTAALGCLVKDYFPEPVTVSWNSGALTSGVHTFPAVLQSSGLYSLSSVVTVPSSSLGTKTYTCNVDHKPSNTKVDKRVESKYGPPCPPCPAPEFLGGPSVFLFPPKPKDTLMISRTPEVTCVVVDVSQEDPEVQFNWYVDGVEVHNAKTKPREEQFNSTYRVVSVLTVLHQDWLNGKEYKCKVSNKGLPSSIEKTISKAKGQPREPQVYTLPPSQEEMTKNQVSLTCLVKGFYPSDIAVEWESNGQPENNYKTTPPVLDSDGSFFLYSRLTVDKSRWQEGNVFSCSVMHEALHNHYTQKSLSLSLGK

SEQ ID NO: 12 - protein, 215 aa, synthetic construct
EIVLTQSPGTLSLSPGERATLSCRASQSVRGRYLAWYQQKPGQAPRLLIYGASSRATGIPDRFSGSGSGTDFTLTISRLEPEDFAVFYCQQYGSSPRTFGQGTKVEIKRTVAAPSVFIFPPSDEQLKSGTASVVCLLNNFYPREAKVQWKVDNALQSGNSQESVTEQDSKDSTYSLSSTLTLSKADYEKHKVYACEVTHQGLSSPVTKSFNRGEC

SEQ ID NO: 13 - protein, 448 aa, synthetic construct
EVQLLESGGGLVQPGGSLRLSCAASGFTFSSYAMSWVRQAPGKGLEWVSGITGSGGSTYYADSVKGRFTISRDNSKNTLYLQMNSLRAEDTAVYYCAKDPGTTVIMSWFDPWGQGTLVTVSSASTKGPSVFPLAPCSRSTSESTAALGCLVKDYFPEPVTVSWNSGALTSGVHTFPAVLQSSGLYSLSSVVTVPSSNFGTQTYTCNVDHKPSNTKVDKTVERKCCVECPPCPAPPVAGPSVFLFPPKPKDTLMISRTPEVTCVVVDVSHEDPEVQFNWYVDGVEVHNAKTKPREEQFNSTFRVVSVLTVVHQDWLNGKEYKCKVSNKGLPAPIEKTISKTKGQPREPQVYTLPPSREEMTKNQVSLTCLVKGFYPSDIAVEWESNGQPENNYKTTPPMLDSDGSFFLYSKLTVDKSRWQQGNVFSCSVMHEALHNHYTQKSLSLSPGK

SEQ ID NO: 14 - protein, 215 aa, synthetic construct; identical to SEQ ID NO: 12

SEQ ID NO: 15 - protein, 5 aa, synthetic construct
GYDLN

SEQ ID NO: 16 - protein, 16 aa, synthetic construct
IIWGDGTTDYNSAVKS

SEQ ID NO: 17 - protein, 13 aa, synthetic construct
GGYWYATSYYFDY

SEQ ID NO: 18 - protein, 11 aa, synthetic construct
RASQSISNNLN

SEQ ID NO: 19 - protein, 7 aa, synthetic construct
YTSRFHS

SEQ ID NO: 20 - protein, 9 aa, synthetic construct
QQEHTLPYT

SEQ ID NO: 21 - protein, 121 aa, synthetic construct [sequence omitted]

SEQ ID NO: 22 - protein, 107 aa, synthetic construct [sequence omitted]

SEQ ID NO: 23 - protein, 326 aa, synthetic construct
ASTKGPSVFPLAPCSRSTSESTAALGCLVKDYFPEPVTVSWNSGALTSGVHTFPAVLQSSGLYSLSSVVTVPSSNFGTQTYTCNVDHKPSNTKVDKTVERKCCVECPPCPAPPVAGPSVFLFPPKPKDTLMISRTPEVTCVVVDVSHEDPEVQFNWYVDGVEVHNAKTKPREEQFNSTFRVVSVLTVVHQDWLNGKEYKCKVSNKGLPSSIEKTISKTKGQPREPQVYTLPPSREEMTKNQVSLTCLVKGFYPSDIAVEWESNGQPENNYKTTPPMLDSDGSFFLYSKLTVDKSRWQQGNVFSCSVMHEALHNHYTQKSLSLSPGK

SEQ ID NO: 24 - protein, 448 aa, synthetic construct
QVQLQESGPGLVKPSETLSLTCTVSGFSLIGYDLNWIRQPPGKGLEWIGIIWGDGTTDYNSAVKSRVTISKDTSKNQFSLKLSSVTAADTAVYYCARGGYWYATSYYFDYWGQGTLVTVSSASTKGPSVFPLAPCSRSTSESTAALGCLVKDYFPEPVTVSWNSGALTSGVHTFPAVLQSSGLYSLSSVVTVPSSSLGTKTYTCNVDHKPSNTKVDKRVESKYGPPCPPCPAPEFLGGPSVFLFPPKPKDTLMISRTPEVTCVVVDVSQEDPEVQFNWYVDGVEVHNAKTKPREEQFNSTYRVVSVLTVLHQDWLNGKEYKCKVSNKGLPSSIEKTISKAKGQPREPQVYTLPPSQEEMTKNQVSLTCLVKGFYPSDIAVEWESNGQPENNYKTTPPVLDSDGSFFLYSRLTVDKSRWQEGNVFSCSVMHEALHNHYTQKSLSLSLGK

SEQ ID NO: 25 - protein, 214 aa, synthetic construct
DIQMTQSPSSLSASVGDRVTITCRASQSISNNLNWYQQKPGKAPKLLIYYTSRFHSGVPSRFSGSGSGTDFTFTISSLQPEDIATYYCQQEHTLPYTFGQGTKLEIKRTVAAPSVFIFPPSDEQLKSGTASVVCLLNNFYPREAKVQWKVDNALQSGNSQESVTEQDSKDSTYSLSSTLTLSKADYEKHKVYACEVTHQGLSSPVTKSFNRGEC

SEQ ID NO: 26 - protein, 447 aa, synthetic construct
QVQLQESGPGLVKPSETLSLTCTVSGFSLIGYDLNWIRQPPGKGLEWIGIIWGDGTTDYNSAVKSRVTISKDTSKNQFSLKLSSVTAADTAVYYCARGGYWYATSYYFDYWGQGTLVTVSSASTKGPSVFPLAPCSRSTSESTAALGCLVKDYFPEPVTVSWNSGALTSGVHTFPAVLQSSGLYSLSSVVTVPSSNFGTQTYTCNVDHKPSNTKVDKTVERKCCVECPPCPAPPVAGPSVFLFPPKPKDTLMISRTPEVTCVVVDVSHEDPEVQFNWYVDGVEVHNAKTKPREEQFNSTFRVVSVLTVVHQDWLNGKEYKCKVSNKGLPSSIEKTISKTKGQPREPQVYTLPPSREEMTKNQVSLTCLVKGFYPSDIAVEWESNGQPENNYKTTPPMLDSDGSFFLYSKLTVDKSRWQQGNVFSCSVMHEALHNHYTQKSLSLSPGK

SEQ ID NO: 27 - protein, 214 aa, synthetic construct; identical to SEQ ID NO: 25

SEQ ID NO: 28 - protein, 6 aa, synthetic construct
ASTKGP

SEQ ID NO: 29 - protein, 5 aa, synthetic construct
TVAAP

SEQ ID NO: 30 - protein, 576 aa, synthetic construct
EVQLLESGGGLVQPGGSLRLSCAASGFTFSSYAMSWVRQAPGKGLEWVSGITGSGGSTYYADSVKGRFTISRDNSKNTLYLQMNSLRAEDTAVYYCVKDPGTTSIMSWFDPWGQGTLVTVSSASTKGPQVQLQESGPGLVKPSETLSLTCTVSGFSLIGYDLNWIRQPPGKGLEWIGIIWGDGTTDYNSAVKSRVTISKDTSKNQFSLKLSSVTAADTAVYYCARGGYWYATSYYFDYWGQGTLVTVSSASTKGPSVFPLAPCSRSTSESTAALGCLVKDYFPEPVTVSWNSGALTSGVHTFPAVLQSSGLYSLSSVVTVPSSSLGTKTYTCNVDHKPSNTKVDKRVESKYGPPCPPCPAPEFLGGPSVFLFPPKPKDTLMISRTPEVTCVVVDVSQEDPEVQFNWYVDGVEVHNAKTKPREEQFNSTYRVVSVLTVLHQDWLNGKEYKCKVSNKGLPSSIEKTISKAKGQPREPQVYTLPPSQEEMTKNQVSLTCLVKGFYPSDIAVEWESNGQPENNYKTTPPVLDSDGSFFLYSRLTVDKSRWQEGNVFSCSVMHEALHNHYTQKSLSLSLGK

SEQ ID NO: 31 - protein, 327 aa, synthetic construct
EIVLTQSPGTLSLSPGERATLSCRASQSVRGRYLAWYQQKPGQAPRLLIYGASSRATGIPDRFSGSGSGTDFTLTISRLEPEDFAVFYCQQYGSSPRTFGQGTKVEIKTVAAPDIQMTQSPSSLSASVGDRVTITCRASQSISNNLNWYQQKPGKAPKLLIYYTSRFHSGVPSRFSGSGSGTDFTFTISSLQPEDIATYYCQQEHTLPYTFGQGTKLEIKRTVAAPSVFIFPPSDEQLKSGTASVVCLLNNFYPREAKVQWKVDNALQSGNSQESVTEQDSKDSTYSLSSTLTLSKADYEKHKVYACEVTHQGLSSPVTKSFNRGEC

SEQ ID NO: 32 - protein, 5 aa, synthetic construct
DYDMS

SEQ ID NO: 33 - protein, 17 aa, synthetic construct
WIYPSGGSIYYADSVKG

SEQ ID NO: 34 - protein, 18 aa, synthetic construct
SGLTRTRWPIYYADGMDV

SEQ ID NO: 35 - protein, 13 aa, synthetic construct
TGSSSNIGNNAVS

SEQ ID NO: 36 - protein, 7 aa, synthetic construct
SDRHRPS

SEQ ID NO: 37 - protein, 11 aa, synthetic construct
GSWDASLSGYV

SEQ ID NO: 38 - protein, 127 aa, synthetic construct
EVQLLESGGGLVQPGGSLRLSCAASGFTFSDYDMSWVRQAPGKGLEWVSWIYPSGGSIYYADSVKGRFTISRDNSKNTLYLQMNSLRAEDTAVYYCARSGLTRTRWPIYYADGMDVWGQGTLVTVSS

SEQ ID NO: 39 - protein, 110 aa, synthetic construct
QSVLTQPPSASGTPGQRVTISCTGSSSNIGNNAVSWYQQLPGTAPKLLIYSDRHRPSGVPDRFSGSKSGTSASLAISGLRSEDEADYYCGSWDASLSGYVFGGGTKLTVL

SEQ ID NO: 40 - protein, 454 aa, synthetic construct
EVQLLESGGGLVQPGGSLRLSCAASGFTFSDYDMSWVRQAPGKGLEWVSWIYPSGGSIYYADSVKGRFTISRDNSKNTLYLQMNSLRAEDTAVYYCARSGLTRTRWPIYYADGMDVWGQGTLVTVSSASTKGPSVFPLAPCSRSTSESTAALGCLVKDYFPEPVTVSWNSGALTSGVHTFPAVLQSSGLYSLSSVVTVPSSSLGTKTYTCNVDHKPSNTKVDKRVESKYGPPCPPCPAPEFLGGPSVFLFPPKPKDTLMISRTPEVTCVVVDVSQEDPEVQFNWYVDGVEVHNAKTKPREEQFNSTYRVVSVLTVLHQDWLNGKEYKCKVSNKGLPSSIEKTISKAKGQPREPQVYTLPPSQEEMTKNQVSLTCLVKGFYPSDIAVEWESNGQPENNYKTTPPVLDSDGSFFLYSRLTVDKSRWQEGNVFSCSVMHEALHNHYTQKSLSLSLGK

SEQ ID NO: 41 - protein, 216 aa, synthetic construct
QSVLTQPPSASGTPGQRVTISCTGSSSNIGNNAVSWYQQLPGTAPKLLIYSDRHRPSGVPDRFSGSKSGTSASLAISGLRSEDEADYYCGSWDASLSGYVFGGGTKLTVLGQPKANPTVTLFPPSSEELQANKATLVCLISDFYPGAVTVAWKADGSPVKAGVETTKPSKQSNNKYAASSYLSLTPEQWKSHRSYSCQVTHEGSTVEKTVAPTECS